European Patent Application EP 4 488 395 A2, published January 8, 2025. Title: PROXIMITY-BASED LABELING SYSTEMS AND APPLICATIONS THEREOF. Applicant: THE TRUSTEES OF PRINCETON UNIVERSITY. Application EP EP 20819012.4, filed November 17, 2021. The sequence listing filed with the application follows.

SEQUENCE LISTING (6 sequences)

SEQ ID NO: 1 - protein, 15 aa, synthetic construct
  MOD_RES 1: note = Lys-Iridium photocatalytic complex
  MOD_RES 5: note = Cycloalkyl-alanine
  MOD_RES 11: note = Alkene alanine
  MOD_RES 12: note = Cycloalkyl-alanine
  REGION 1..15: note = source = /note="Description of Artificial Sequence: Synthetic peptide"
  REGION 1..15: note = source = /note="ATSP7041"
XLTFXEYWAQXXSAA

SEQ ID NO: 2 - protein, 31 aa, synthetic construct
  REGION 1..31: note = source = /note="Description of Artificial Sequence: Synthetic polypeptide"
PFKFMLGKQEVIRGWEEGVAQMSVGQRAKLT

SEQ ID NO: 3 - protein, 26 aa, synthetic construct
  REGION 1..26: note = source = /note="Description of Artificial Sequence: Synthetic peptide"
AEIYAYREEQEYGIETVKVKAIGRQR

SEQ ID NO: 4 - protein, 21 aa, synthetic construct
  REGION 1..21: note = source = /note="Description of Artificial Sequence: Synthetic peptide"
RFVNLMKESFETFINKRPNKP

SEQ ID NO: 5 - protein, 41 aa, synthetic construct
  REGION 1..41: note = source = /note="Description of Artificial Sequence: Synthetic polypeptide"
SFELKFLEETNCLYAAEGQRLMQEREVPEYLNHVSKRLEEE

SEQ ID NO: 6 - protein, 41 aa, synthetic construct
  REGION 1..41: note = source = /note="Description of Artificial Sequence: Synthetic polypeptide"
IKNFRDRPRLPDNYTQDTWRKLHEAVRAVQSSTSIRYNEEE